European Patent Specification EP 3 622 064 B1, published May 14, 2025. Title: MANNANASE VARIANTS AND POLYNUCLEOTIDES ENCODING SAME. Applicant: Novozymes A/S. The sequence listing filed with the application follows.

SEQUENCE LISTING (3 sequences)

SEQ ID NO: 1 - protein, 326 aa, Bacillus bogoriensis
  mat_peptide (29)..(326)
MKQQKRLYARLLTLLFALIFLLPHSAAAANSGFYVSGTTLYDANGNPFVMRGINHGHAWYKDQATTAIEGIANTGANTVRIVLSDGGQWTKDDIHTVRNLISLAEDNHLVAVLEVHDATGYDSIASLNRAVDYWIEMRSALIGKEDTVIINIANEWFGSWEGDAWADGYKQAIPRLRNAGLNHTLMVDAAGWGQFPQSIHDYGREVFNADPQRNTMFSIHMYEYAGGNASQVRTNIDRVLNQDLALVIGEFGHRHTNGDVDEATIMSYSEQRGVGWLAWSWKGNGPEWEYLDLSNDWAGNNLTAWGNTIVNGPYGLRETSRLSTVF

SEQ ID NO: 2 - protein, 298 aa, Bacillus bogoriensis
ANSGFYVSGTTLYDANGNPFVMRGINHGHAWYKDQATTAIEGIANTGANTVRIVLSDGGQWTKDDIHTVRNLISLAEDNHLVAVLEVHDATGYDSIASLNRAVDYWIEMRSALIGKEDTVIINIANEWFGSWEGDAWADGYKQAIPRLRNAGLNHTLMVDAAGWGQFPQSIHDYGREVFNADPQRNTMFSIHMYEYAGGNASQVRTNIDRVLNQDLALVIGEFGHRHTNGDVDEATIMSYSEQRGVGWLAWSWKGNGPEWEYLDLSNDWAGNNLTAWGNTIVNGPYGLRETSRLSTVF

SEQ ID NO: 3 - DNA, 981 bp, Bacillus bogoriensis
atgaaacaacaaaaacggctttacgcccgattgctgacgctgttatttgcgctcatcttcttgctgcctcattctgcagccgcggcaaattccggattttatgtaagcggtaccactctatacgatgccaatggaaacccatttgtaatgagagggattaaccatgggcacgcatggtataaagaccaggcaactactgcaattgaagggattgcaaataccggtgctaatacggtccggattgtgttatctgatgggggacaatggacaaaagatgacatccatacagtaagaaaccttatctctttagcggaagataatcatttggttgctgttcttgaagttcatgatgctaccggttatgattccattgcttcgctcaatcgtgctgttgattattggattgaaatgagaagtgctttaattggaaaggaagataccgtcattattaatattgcgaatgaatggtttggttcgtgggaaggggatgcttgggctgacgggtataaacaagcaatcccgcgattgcgtaacgccggtctaaaccataccttgatggtagatgctgcggggtggggacaatttccacaatcgattcatgattatggaagagaagtttttaatgctgaccctcaacgaaatacaatgttttcgattcatatgtatgaatatgcaggtggtaatgcatcgcaagttcgtactaatattgaccgagttcttaatcaagacctcgcattagtcattggtgaatttggacaccgtcatacaaatggtgacgtcgatgaagcaacgattatgagctattctgaacaaagaggagttgggtggttggcgtggtcatggaaagggaacggcccagaatgggagtatttagacctttcgaatgattgggctggaaataaccttacagcttggggaaatacaatagtgaatggtccatatggtttaagagaaacttcgagattaagcaccgttttttga